European Patent Application EP 4 410 372 A1, published August 7, 2024. Title: An antibody and antibody-drug conjugate and use thereof. Applicant: EVOPOINT BIOSCIENCES CO., LTD. The sequence listing filed with the application follows.

SEQUENCE LISTING (53 sequences)

SEQ ID NO: 1 - protein, 117 aa, artificial sequence
QVQLVQSGAEVKKPGSSVKVSCKASGYTFTNYWLHWVRQAPGQGLEWMGMMHPISGSSNYAQKFQGRATLTVDKSTSTAYMELSSLRSEDTAVYYCARGLLSAMDYWGQGTLVTVSS

SEQ ID NO: 2 - protein, 107 aa, artificial sequence
EIVLTQSPATLSLSPGERATLSCKASENVKTYVSWYQQKPGQSPRLLIYEASNRYTGVPARFSGSGSATDFTLTISSLEPEDFAVYFCGQTYSFPPTFGQGTKVEIK

SEQ ID NO: 3 - protein, 117 aa, artificial sequence
QVQLVESGAEVKKPGSSVKVSCKASGYTFTNYWLHWVRQAPGQGLEWMGMMHPISGSSNYAQKFQGRATLTVDKSTSTAYMELSSLRSEDTAVYYCARGLLSAMDYWGQGTLVTVSS

SEQ ID NO: 4 - protein, 330 aa, artificial sequence [sequence omitted]

SEQ ID NO: 5 - protein, 107 aa, artificial sequence [sequence omitted]

SEQ ID NO: 6 - protein, 8 aa, artificial sequence
GYTFTNYW

SEQ ID NO: 7 - protein, 8 aa, artificial sequence
MHPISGSS

SEQ ID NO: 8 - protein, 10 aa, artificial sequence
ARGLLSAMDY

SEQ ID NO: 9 - protein, 6 aa, artificial sequence
ENVKTY

SEQ ID NO: 10 - skipped

SEQ ID NO: 11 - protein, 9 aa, artificial sequence
GQTYSFPPT

SEQ ID NO: 12 - protein, 5 aa, artificial sequence
NYWLH

SEQ ID NO: 13 - protein, 17 aa, artificial sequence
MMHPISGSSNYAQKFQG

SEQ ID NO: 14 - protein, 8 aa, artificial sequence
GLLSAMDY

SEQ ID NO: 15 - protein, 11 aa, artificial sequence
KASENVKTYVS

SEQ ID NO: 16 - protein, 7 aa, artificial sequence
EASNRYT

SEQ ID NO: 17 - protein, 9 aa, artificial sequence
GQTYSFPPT

SEQ ID NO: 18 - protein, 447 aa, artificial sequence
QVQLVQSGAEVKKPGSSVKVSCKASGYTFTNYWLHWVRQAPGQGLEWMGMMHPISGSSNYAQKFQGRATLTVDKSTSTAYMELSSLRSEDTAVYYCARGLLSAMDYWGQGTLVTVSSASTKGPSVFPLAPSSKSTSGGTAALGCLVKDYFPEPVTVSWNSGALTSGVHTFPAVLQSSGLYSLSSVVTVPSSSLGTQTYICNVNHKPSNTKVDKKVEPKSCDKTHTCPPCPAPELLGGPSVFLFPPKPKDTLMISRTPEVTCVVVDVSHEDPEVKFNWYVDGVEVHNAKTKPREEQYNSTYRVVSVLTVLHQDWLNGKEYKCKVSNKALPAPIEKTISKAKGQPREPQVYTLPPSRDELTKNQVSLTCLVKGFYPSDIAVEWESNGQPENNYKTTPPVLDSDGSFFLYSKLTVDKSRWQQGNVFSCSVMHEALHNHYTQKSLSLSPGK

SEQ ID NO: 19 - protein, 447 aa, artificial sequence
QVQLVESGAEVKKPGSSVKVSCKASGYTFTNYWLHWVRQAPGQGLEWMGMMHPISGSSNYAQKFQGRATLTVDKSTSTAYMELSSLRSEDTAVYYCARGLLSAMDYWGQGTLVTVSSASTKGPSVFPLAPSSKSTSGGTAALGCLVKDYFPEPVTVSWNSGALTSGVHTFPAVLQSSGLYSLSSVVTVPSSSLGTQTYICNVNHKPSNTKVDKKVEPKSCDKTHTCPPCPAPELLGGPSVFLFPPKPKDTLMISRTPEVTCVVVDVSHEDPEVKFNWYVDGVEVHNAKTKPREEQYNSTYRVVSVLTVLHQDWLNGKEYKCKVSNKALPAPIEKTISKAKGQPREPQVYTLPPSRDELTKNQVSLTCLVKGFYPSDIAVEWESNGQPENNYKTTPPVLDSDGSFFLYSKLTVDKSRWQQGNVFSCSVMHEALHNHYTQKSLSLSPGK

SEQ ID NO: 20 - protein, 214 aa, artificial sequence
EIVLTQSPATLSLSPGERATLSCKASENVKTYVSWYQQKPGQSPRLLIYEASNRYTGVPARFSGSGSATDFTLTISSLEPEDFAVYFCGQTYSFPPTFGQGTKVEIKRTVAAPSVFIFPPSDEQLKSGTASVVCLLNNFYPREAKVQWKVDNALQSGNSQESVTEQDSKDSTYSLSSTLTLSKADYEKHKVYACEVTHQGLSSPVTKSFNRGEC

SEQ ID NO: 21 - protein, 117 aa, artificial sequence
EVQLQQPGAELVKPGTSVKLSCKASGYTFTNYWLHWVRQRPGQGLEWIGMMHPISGSSNNNERFKSKATLTVDKSSTTAYMQLSRMTSEDSAVYYCARGLLSAMDYWGQGTSVTVSS

SEQ ID NO: 22 - protein, 107 aa, artificial sequence
CIVLTQSPKSMSMSVGERVTLSCKASENVKTYVSWYQQRPEQSPKLLIYEASNRYTGVPDRFTGSGSATVFTLTISSVQTEDLANYFCGQTYSFPPTFGSGTKLEIK

SEQ ID NO: 23 - protein, 118 aa, artificial sequence
EVQLQQSGPELVKPGASVRMSCKASGYTFTSYVVHWVKQKPGQGLEWIGYINPYNADSKYNERFKGKATLTSDKSSNSAYMELSSLTSEDSAVYYCSRSYYGNSFDVWGAGTTVTVSS

SEQ ID NO: 24 - protein, 113 aa, artificial sequence
DIVMTQSPSSLTVTTGEKVTMSCKSSQSLLNSGNQKNYLTWYQQKPGQSPKLLFFWASTRQSGVPDRFTGSGSGTYFTLTISSVQAEDLAVYYCQNDYYFPFTFGTGTKLEIK

SEQ ID NO: 25 - protein, 17 aa, artificial sequence
MMHPISGSSNNNERFKS

SEQ ID NO: 26 - protein, 5 aa, artificial sequence
SYVVH

SEQ ID NO: 27 - protein, 17 aa, artificial sequence
YINPYNADSKYNERFKG

SEQ ID NO: 28 - protein, 9 aa, artificial sequence
SYYGNSFDV

SEQ ID NO: 29 - protein, 8 aa, artificial sequence
GYTFTSYV

SEQ ID NO: 30 - protein, 8 aa, artificial sequence
INPYNADS

SEQ ID NO: 31 - protein, 11 aa, artificial sequence
SRSYYGNSFDV

SEQ ID NO: 32 - protein, 17 aa, artificial sequence
KSSQSLLNSGNQKNYLT

SEQ ID NO: 33 - protein, 7 aa, artificial sequence
WASTRQS

SEQ ID NO: 34 - protein, 9 aa, artificial sequence
QNDYYFPFT

SEQ ID NO: 35 - protein, 12 aa, artificial sequence
QSLLNSGNQKNY

SEQ ID NO: 36 - skipped

SEQ ID NO: 37 - protein, 17 aa, artificial sequence
YINPYNADSKYSQEFQG

SEQ ID NO: 38 - protein, 118 aa, artificial sequence
QVQLVQSGAEVKKPGASVKVSCKASGYTFTSYVVHWVRQAPGQGLEWMGYINPYNADSKYSQEFQGRATLTSDKSASTAYMELSSLRSEDMAVYYCSRSYYGNSFDVWGQGTLVTVSS

SEQ ID NO: 39 - protein, 113 aa, artificial sequence
DIVMTQSPDSLAVSLGERATINCKSSQSLLNSGNQKNYLTWYQQKPGQSPKLLFFWASTRQSGVPDRFSGSGSGTDFTLTISSLQAEDVAVYYCQNDYYFPFTFGQGTKVEIK

SEQ ID NO: 40 - protein, 118 aa, artificial sequence
QVQLVESGAEVKKPGASVKVSCKASGYTFTSYVVHWVRQAPGQGLEWMGYINPYNADSKYSQEFQGRATLTSDKSASTAYMELSSLRSEDMAVYYCSRSYYGNSFDVWGQGTLVTVSS

SEQ ID NO: 41 - protein, 448 aa, artificial sequence
QVQLVQSGAEVKKPGASVKVSCKASGYTFTSYVVHWVRQAPGQGLEWMGYINPYNADSKYSQEFQGRATLTSDKSASTAYMELSSLRSEDMAVYYCSRSYYGNSFDVWGQGTLVTVSSASTKGPSVFPLAPSSKSTSGGTAALGCLVKDYFPEPVTVSWNSGALTSGVHTFPAVLQSSGLYSLSSVVTVPSSSLGTQTYICNVNHKPSNTKVDKKVEPKSCDKTHTCPPCPAPELLGGPSVFLFPPKPKDTLMISRTPEVTCVVVDVSHEDPEVKFNWYVDGVEVHNAKTKPREEQYNSTYRVVSVLTVLHQDWLNGKEYKCKVSNKALPAPIEKTISKAKGQPREPQVYTLPPSRDELTKNQVSLTCLVKGFYPSDIAVEWESNGQPENNYKTTPPVLDSDGSFFLYSKLTVDKSRWQQGNVFSCSVMHEALHNHYTQKSLSLSPGK

SEQ ID NO: 42 - protein, 448 aa, artificial sequence
QVQLVESGAEVKKPGASVKVSCKASGYTFTSYVVHWVRQAPGQGLEWMGYINPYNADSKYSQEFQGRATLTSDKSASTAYMELSSLRSEDMAVYYCSRSYYGNSFDVWGQGTLVTVSSASTKGPSVFPLAPSSKSTSGGTAALGCLVKDYFPEPVTVSWNSGALTSGVHTFPAVLQSSGLYSLSSVVTVPSSSLGTQTYICNVNHKPSNTKVDKKVEPKSCDKTHTCPPCPAPELLGGPSVFLFPPKPKDTLMISRTPEVTCVVVDVSHEDPEVKFNWYVDGVEVHNAKTKPREEQYNSTYRVVSVLTVLHQDWLNGKEYKCKVSNKALPAPIEKTISKAKGQPREPQVYTLPPSRDELTKNQVSLTCLVKGFYPSDIAVEWESNGQPENNYKTTPPVLDSDGSFFLYSKLTVDKSRWQQGNVFSCSVMHEALHNHYTQKSLSLSPGK

SEQ ID NO: 43 - protein, 220 aa, artificial sequence
DIVMTQSPDSLAVSLGERATINCKSSQSLLNSGNQKNYLTWYQQKPGQSPKLLFFWASTRQSGVPDRFSGSGSGTDFTLTISSLQAEDVAVYYCQNDYYFPFTFGQGTKVEIKRTVAAPSVFIFPPSDEQLKSGTASVVCLLNNFYPREAKVQWKVDNALQSGNSQESVTEQDSKDSTYSLSSTLTLSKADYEKHKVYACEVTHQGLSSPVTKSFNRGEC

SEQ ID NO: 44 - protein, 116 aa, artificial sequence
QVQLKESGPVLVAPSQSLSITCTVSGFSLTNYGVHWVRQPPGKGLEWLGVIWSGGRTNYNSALMSRLSISKDNSKSQVFLKMNSLQTDDTAMYYCAKRDGIYGDYWGQGTSVTVSS

SEQ ID NO: 45 - protein, 113 aa, artificial sequence
DIVETQSPSSLTVTAGEKVTMSCKSSQSLLNSGNQKNYLTWYQQKPGQSPKLLIYWASTRESGVPDRFTGSGFGTDFTLTISSVQAEDLAVYYCQNDYIYPLTFGAGTKLELK

SEQ ID NO: 46 - protein, 118 aa, artificial sequence
QVQLKESGGGLVKPGGSLKLSCAASGFTFSSYAMSWVRQTPEKRLEWVAAIHSNGGSTYNSDTMRDRFTISRDHAKNTLYLQMSSLRSEDTALYYCGRQSFGNALDYWGQGTSVTVSS

SEQ ID NO: 47 - protein, 113 aa, artificial sequence
DIQMTQSPSSLTVTAGEKVTLTCKSSQSLLNSGNQKNYLTWYQQKPGQPPKLLIYWASTRESGVPDRFTGSGSGTFFTLTISSVQAEDLAVYFCQNDYVYPFTFGAGTQLELK

SEQ ID NO: 48 - protein, 119 aa, artificial sequence
QVQLKESGGGLVQPGGSMKLSCAASGFTFSDAWMNWVRQSPEKGLEWVAEIRNKADYHATHYVESVTGRFTISRDDSKSSVYLQMNRLRAEDTGIYYCTRNYGSRFDYWGQGTTLTVSS

SEQ ID NO: 49 - protein, 113 aa, artificial sequence
DIVETQSPSSLTVTAGEKVTMSCKSSQSLLNSGNQRNYLTWYQQKPGHPPKLLIYWASTRESGVPDRFTGSGSGTDFTLTVTSVQAEDLAVYYCQNDYFYPLAFGTGTKLELK

SEQ ID NO: 50 - protein, 118 aa, artificial sequence
EVQLQQSGAELARPGASVKLSCKASGYTFTSYGIRWVKQRTGQGLEWIGEIYPRGGNTYYDEKFKGKATLTADKSSSTAYMGLRSLTSEDSAVYFCARADYGNSFAYWGQGTLVTVSA

SEQ ID NO: 51 - protein, 113 aa, artificial sequence
DIVMTQSPSSLTVTAREKVTMSCKSSQSLLNSGNQKNYLTWYHQKPGQPPKLLIYWASTRESGVPDRFTGSGSGTDFTLTISSVQAEDLAVYFCQNAYFYPFTFGTGTKLEIK

SEQ ID NO: 52 - protein, 118 aa, artificial sequence
QIQLVQSGPELRKPGETVKISCKASGYTFTAYTMGWVKQAPGKGLEWMAWINTYSGVPTYAADFKGRFAFSLETSASTAYLLINNLKNEDTATYFCARGVRGNSMDYWGQGTSVTVSS

SEQ ID NO: 53 - protein, 113 aa, artificial sequence
DIVETQSPSSLTVTVGERVTLSCKSSQSLLNSGNQRNYLTWSQQKPGQPPKLLIYWASTRESGVPNRFTGGGSGTYFTLTISSVQVEDLAVYYCQNTYSFPFTFGTGTKLEIK